European Patent Application EP 4 289 864 A1, published December 13, 2023. Title: METHOD FOR INHIBITING TUMOUR CELL GROWTH BASED ON CCDC112. Applicant: BIOTROY THERAPEUTICS. The sequence listing filed with the application follows.

SEQUENCE LISTING (35 sequences)

SEQ ID NO: 1 - DNA, 20 bp, Artificial Sequence
cacttctacatatcccacat

SEQ ID NO: 2 - DNA, 20 bp, Artificial Sequence
ggtgggtttgtaaagcctag

SEQ ID NO: 3 - DNA, 20 bp, Artificial Sequence
ctggtgatcataatcatccc

SEQ ID NO: 4 - DNA, 20 bp, Artificial Sequence
tccaggttggaatagcccta

SEQ ID NO: 5 - DNA, 20 bp, Artificial Sequence
aattctagatagacaggcaa

SEQ ID NO: 6 - DNA, 20 bp, Artificial Sequence
tttacaaacccaccaaaggt

SEQ ID NO: 7 - DNA, 20 bp, Artificial Sequence
tgtttattatgaaaaagcac

SEQ ID NO: 8 - DNA, 20 bp, Artificial Sequence
taaaaagcagcaaaaaaggg

SEQ ID NO: 9 - DNA, 1341 bp, Artificial Sequence
atggaaaaagataaacacagtcatttctacaaccaaaaaagtgacttcagaattgagcatagtatgctagaagaattggaaaataaattgattcacagcaggaaaacagaaagagcaaaaatccagcaacaattggccaaaatacataataatgtaaagaaacttcagcatcaattaaaagatgtgaagcctacacctgattttgttgagaagctcagagaaatgatggaagaaattgaaaatgcaattaacacttttaaagaagagcagaggttgatatatgaagagctaattaaagaagagaagacaactaataatgagttgagtgccatatcaagaaaaattgacacatgggctttgggtaattcagaaacagagaaagctttcagagcaatctcaagcaaagttcctgtagacaaagtaacaccaagtactcttccagaagaggtactagattttgaaaaattccttcagcaaacaggagggcgacaaggtgcctgggatgattatgatcaccagaactttgtaaaggtgagaaacaaacataaagggaagccaacatttatggaagaagttctagaacaccttcctggaaaaacacaagatgaagttcaacagcatgaaaaatggtatcaaaagtttctggctctagaagaaagaaaaaaagagtcaattcagatttggaaaactaaaaagcagcaaaaaagggaggaaattttcaagttaaaggaaaaggcagacaacacacctgtgctttttcataataaacaagaggataatcaaaagcaaaaagaggaacaaagaaagaaacagaaattggcagttgaagcttggaagaaacagaaaagtatagaaatgtcaatgaaatgtgcttcccagttaaaagaagaagaagagaaagagaaaaaacatcagaaagaacgccagcgccagtttaagttaaaattactactagaaagttatacccagcagaagaaagaacaggaagaatttttgaggcttgaaaaggagataagggaaaaggcagaaaaggcagaaaaaaggaaaaatgctgctgatgaaatttccagatttcaagaaagagatttacataaacttgaactgaaaattctagatagacaggcaaaggaagatgaaaagtcacaaaaacaaagaagactggcaaaattaaaagaaaaggttgaaaacaatgttagtagagatccctctaggctttacaaacccaccaaaggttgggaagaacgaaccaaaaagataggaccaacaggctctgggccacttctacatatcccacatagggctattccaacctggagacaaggaatacagagaagagtatga

SEQ ID NO: 10 - protein, 446 aa, Artificial Sequence
MEKDKHSHFYNQKSDFRIEHSMLEELENKLIHSRKTERAKIQQQLAKIHNNVKKLQHQLKDVKPTPDFVEKLREMMEEIENAINTFKEEQRLIYEELIKEEKTTNNELSAISRKIDTWALGNSETEKAFRAISSKVPVDKVTPSTLPEEVLDFEKFLQQTGGRQGAWDDYDHQNFVKVRNKHKGKPTFMEEVLEHLPGKTQDEVQQHEKWYQKFLALEERKKESIQIWKTKKQQKREEIFKLKEKADNTPVLFHNKQEDNQKQKEEQRKKQKLAVEAWKKQKSIEMSMKCASQLKEEEEKEKKHQKERQRQFKLKLLLESYTQQKKEQEEFLRLEKEIREKAEKAEKRKNAADEISRFQERDLHKLELKILDRQAKEDEKSQKQRRLAKLKEKVENNVSRDPSRLYKPTKGWEERTKKIGPTGSGPLLHIPHRAIPTWRQGIQRRV

SEQ ID NO: 11 - DNA, 342 bp, Artificial Sequence
caggttcaactgcagcagtctggacctgagctggtgaagcctggggcttcagtgaagataccctgcaagacttctggatactcattcactgactacaacatagactgggtgaagcagggacttggagagagccttgagtggattggagatattaatcctaactatggtggaactatgtacaaccagaagttcaagggcaaggccacattgactgtagacaagtcctccaacacagcctacatggagctccgcagcctgacatctgaagacactgcagtctattactgtgcacatgacgagtttatttactggggccaagggactctggtcactgtctctgca

SEQ ID NO: 12 - DNA, 321 bp, Artificial Sequence
gacatccagatgaaccagtctccatcttccatgtttgcatctctaggagagagagtcactatcacttgcagggcgagtcaggacattaatacctatttaagctggatccagcggaaaccagggaaatctcctaagaccctgatctatcgtgcaaacagattggtagatggggtcccatcaaggttcagtggcagtggatctgggcaagattattctctcaccatcagcagcctggaatatgaagatatgggaatttattattgtctacagtatgatgagtttcctcacacgttcggtggggggaccaagctggaaataaaa

SEQ ID NO: 13 - protein, 114 aa, Artificial Sequence
QVQLQQSGPELVKPGASVKIPCKTSGYSFTDYNIDWVKQGLGESLEWIGDINPNYGGTMYNQKFKGKATLTVDKSSNTAYMELRSLTSEDTAVYYCAHDEFIYWGQGTLVTVSA

SEQ ID NO: 14 - protein, 107 aa, Artificial Sequence
DIQMNQSPSSMFASLGERVTITCRASQDINTYLSWIQRKPGKSPKTLIYRANRLVDGVPSRFSGSGSGQDYSLTISSLEYEDMGIYYCLQYDEFPHTFGGGTKLEIK

SEQ ID NO: 15 - protein, 8 aa, Artificial Sequence
GYSFTDYN

SEQ ID NO: 16 - protein, 8 aa, Artificial Sequence
INPNYGGT

SEQ ID NO: 17 - protein, 7 aa, Artificial Sequence
AHDEFIY

SEQ ID NO: 18 - protein, 6 aa, Artificial Sequence
QDINTY

SEQ ID NO: 19 - protein, 2 aa, Artificial Sequence
RA

SEQ ID NO: 20 - protein, 9 aa, Artificial Sequence
LQYDEFPHT

SEQ ID NO: 21 - protein, 7 aa, Artificial Sequence
GYSFTDY

SEQ ID NO: 22 - protein, 6 aa, Artificial Sequence
NPNYGG

SEQ ID NO: 23 - protein, 5 aa, Artificial Sequence
DEFIY

SEQ ID NO: 24 - protein, 11 aa, Artificial Sequence
RASQDINTYLS

SEQ ID NO: 25 - protein, 7 aa, Artificial Sequence
RANRLVD

SEQ ID NO: 26 - protein, 10 aa, Artificial Sequence
GYSFTDYNID

SEQ ID NO: 27 - protein, 10 aa, Artificial Sequence
DINPNYGGTM

SEQ ID NO: 28 - protein, 5 aa, Artificial Sequence
DYNID

SEQ ID NO: 29 - protein, 17 aa, Artificial Sequence
DINPNYGGTMYNQKFKG

SEQ ID NO: 30 - protein, 6 aa, Artificial Sequence
TDYNID

SEQ ID NO: 31 - protein, 13 aa, Artificial Sequence
WIGDINPNYGGTM

SEQ ID NO: 32 - protein, 6 aa, Artificial Sequence
AHDEFI

SEQ ID NO: 33 - protein, 7 aa, Artificial Sequence
NTYLSWI

SEQ ID NO: 34 - protein, 10 aa, Artificial Sequence
TLIYRANRLV

SEQ ID NO: 35 - protein, 8 aa, Artificial Sequence
LQYDEFPH